European Patent Application EP 4 491 723 A1, published January 15, 2025. Title: 胞嘧啶脱氨酶及其在碱基编辑中的用途. Applicant: 中国科学院遗传与发育生物学研究所. The sequence listing filed with the application follows.

SEQUENCE LISTING (110 sequences)

SEQ ID NO: 1 - protein, 210 aa, synthetic construct
MICKLDSVLMTQKKFIFHYKNVRWARGRHETYLCFVVKRRIGPDSLSFDFGHLRNRSGCHVELLFLRHLGALCPGLSASSVDGARLCYSVTWFCSWSPCSKCAQQLAHFLSQTPNLRLRIFVSRLYFCDEEDSVEREGLRHLKRAGVQISVMTYKDFFYCWQTFVARRERSFKAWDGLHENSVRLVRKLNRILQPCETEDLRDVFALLGL

SEQ ID NO: 2 - protein, 167 aa, synthetic construct
MLDVDDPHTFYVLAGKTPVLVHNSECPIWVKNALQELVGRKETSGKVFDVDGKPIGPDIQSGYKDRELRRGVYETLRKSPFFQKHFPSTATWYVSLHVEAQYAVWMLRNRIKHATVVINNTYVCSDMNRLHDNCMTAVPHILPEGYTMTVWKADRTEVTLRGKAPKE

SEQ ID NO: 3 - protein, 172 aa, synthetic construct
MGPLLDGIAARLEAVRAALLGEGGGAGDDEPPAVPWDRVERLRRELPPPVVPNTGQKTHGRWIGPDGQARPIVSGRDDKSVLVNPLLRGKGAPGPTRRDSDVEMKLAAHMAARGIRHATVVINNTPCRGPLRCDTLVPILLPEGSTLTVHGINENGTRTRIRYTGGARPWWS

SEQ ID NO: 4 - protein, 168 aa, synthetic construct
MLEAVRARLIGEGGGPGAVPEGGDGPPAVPAEEVERLRGELPPPVVPGTGQKTHGRWIGPDGRVRAIVSGRDEDAALVHAQLAAKGIPDEPTRNSDVEQKLAAHMVANGIRHVTLVINHRPCRGFDDSCDTLVPIILPEGCTLTVHGQTDKGMRVRVRYTGGARPWWS

SEQ ID NO: 5 - protein, 212 aa, synthetic construct
MLDAMDAYLSEIAGGNAPARAGPKAPEPKQPGGSSSPRARDGRIDFRALLERLKAQGVVGLEGRSDDPIPDFDPKKQNPACYQGLAPRQKGKPVRGNLFFPDGRRWNDVALESSRGEPAFDLNIIKPEYRSLSPARGHLEGNVAAWMRSTFHQEMVLYINESPCRKHGKGCLYTLEHFLPRGYVLHVWSRNDRGEWRGNTFRGSGEAFTEGA

SEQ ID NO: 6 - protein, 153 aa, synthetic construct
MYVLAGNTPVLVHNTGPGCGEPGFVSDAANSLSGRRITTGQIFDASGNPIGPEITSGGGSLADRAQSYLADSPNIRNLPAKARYASADHVEAQYAVWMRENGVTDASVVINQNYVCGLPLGCQAAVPAILPRGSTMTVWYPGSGSPIVLRGVG

SEQ ID NO: 7 - protein, 226 aa, synthetic construct
MVETRDKIIAAKSRSDAGLLAFQQATNGSIDSRPAEAIANLQRAKTHLDEAQRLVANSDAAVDNYINAILGGASAATAQPSAVIPASKPSRFKPMRTDPAKADEIRPHVGKDRAVATLWDADGNRVLGLHSADDDGPAATAAWKPPWRDYVRLRRHVEAHAAARMHQDGHKTMVMYINLPPCKYFDGCKLNLEDILPKGSTLWMHRVFQNGGTKIYQFNGTGRAYV

SEQ ID NO: 8 - protein, 177 aa, synthetic construct
MPIRLSGGLNLYQYAPETNNWIDPLGCSGHRRRHEKMPPEGARLTTGNLFRHAQDEGISPILSSKNDEFYYRLIKIYAGTGMLNANIRGIASHVEPKAGLILNEDGSGWKIGSLYINYPNGPCLDCRTLMPFILNDGSILYVTFPTLGLDGYSYGHFHGREPGFFREGTPCNLPHPE

SEQ ID NO: 9 - protein, 157 aa, synthetic construct
MADTPQPDSNPLPARDGQRLDREQAEAIRAQLPPTVKPGTGQKTHGCWVDEQGQPQSVTSGQDNSAAAVWARLQALGIPLSGPPTATADVEQKVAIQMIQQGRQHVDVVINNEPCRGRFSCDTLVPIILPEGSSLTVHGTNGFRKTYTGGAKPPWSR

SEQ ID NO: 10 - protein, 115 aa, synthetic construct
MRAGCGVPDGRTRSAISGKDEGFALALRTIRELGMTRGFPLRAADVEMKVASEMRANGITSATLVINHVPCDDGMFSCDRMVPVLLPAGSTLTVFGAGGFRMTYHGGEQLPCPTP

SEQ ID NO: 11 - protein, 167 aa, synthetic construct
MLLTPPPRPAAPPTTRPKPLVARTGDAYPPGTEWALPLIVQPHPPVGGTVPVEGHVRALRPESQISHVFHPGGGHWTEQARARLRVLPGFGWAVNLGHHVELQIAAWMTACGIHHAELVLNRPPCGERYGLGCHQALPVLLPRGYRLTVSSTRGGPQPYQHHYEGKA

SEQ ID NO: 12 - protein, 166 aa, synthetic construct
MLDAALGAVRRIIAALGTSGAERASPGANGSERVDELAERLPPTVVPNTSAKTHGWWFTGQGAAQELISGEGPDARAAYEALREEGYPRPGMPFVAMHVEIKLAAHMRRNDIEHATVVINNIPCPLVWGCENLIGVVLPEGSSLTVHGSNGYERTFTGGRKPPWPR

SEQ ID NO: 13 - protein, 206 aa, synthetic construct
MLGGVLPARSVMFPGHVEPDAHFGPNPERHHPALVEVPIVWAGRQEDRTSTWARRVQRGFPRYTVGAKTAGMFYNAGSQSWELLSGVDHRGGLTRKASQHISRMLSSGFFDGKPLDTKSDHLRMLNYTSTHVETKAAIWARDSDQETIDVVTNRNYVCGESYDPDDVDEPPGCYQAVESVLREGQTMRVWTTDPENRVITIHGKGM

SEQ ID NO: 14 - protein, 160 aa, synthetic construct
MAAGGGVSRPPATRDGAANPTRVPNPPEWLPGWLTEAARDLPRRQAKDPTSGVALINGERIPMRSGRDPAAAADLKAAYKLIATTTDHLEAKLAARMRRDQVMHAEVLTNNPPCDYEPYGCEKILSRLLPAGAQLSVYVRDDDDQVRLWRTYIGNGKAIA

SEQ ID NO: 15 - protein, 162 aa, synthetic construct
MTTGGGSDISRPPATRDTSATATEAPAQPELVPEGLTDAARDLPRRQAKDPTSGVALIGGERIPMRSGRDPDAAADLKPAYKLIATTTDHLEAKLAARMRRDHITQAAVVTNNPPCDYTPYGCEKILSRLLPAGARLAVYVRDDDGQVRHWRTYTGNGKAIA

SEQ ID NO: 16 - protein, 210 aa, synthetic construct
MIRARDRLTAVTASSRHPLVDQALQHVTAAIERLQVADRDAALAASALVAYGRTLGISLPVPPPVSAPTRGAAPVPSWIRQTGQDLPTRPDDHGPTHGQAFDSTGRPLSAEPWRSGRNIASTSDLRPIPGLKGFPWTLTDHVESRAAQQMRRPGAPREVSLVVNKEPCTDDPYGCDRILRHIIPAGSRLTIYVRDPDAPAGVRTVGQYEG

SEQ ID NO: 17 - protein, 208 aa, synthetic construct
MSASAQLNTYLAAIGNSTTTVEAQPEAAPPPAAAESLDSTPRLPDGGIDFHALAKRLGLLEARPTEQPPFDPRRFNPACWQGLKPYDQAGTAEGNLFIAPGKRWNTRPMQASKLEVGPQSDLHPQWRSRKAPWHIEGKIAAYMRQKGFTDGCVYLNARPCSGPDGCARNLPDLLPVGSTLHVHARYIDRTGETRFYYREYRGTGKALT

SEQ ID NO: 18 - protein, 177 aa, synthetic construct
MPIRLSGGLNLYQYAPETNNWIDPLGCSGYRRRHEKMPPEGARLTTGNLFRHAQDEGIPPIFSSENDEFYHRLIEIYAGTGVLNAYIRGIASHVEPKAGLILNEDGSGWKIGSLYINYPDGPCLGCRTLMPFILNDGSILYVTFPTLGLDGYSYGHFHGGVSGFFREGTPCNLRHPE

SEQ ID NO: 19 - protein, 132 aa, synthetic construct
MCGWSELASYRAREGMPARGSADDTFTAARLQIDGQVFFGRNAHGRPVDIRVNAQTKTHAEADVFQQAKDAGATGTRAVLHVVRDFCRSCGATGGVGSLMRGLGVEELLVHSPSGIFTINAVRRPSTPRPLG

SEQ ID NO: 20 - protein, 323 aa, synthetic construct
MRTRPAFGRCDCAGSDRGWEVAGGYTSEASHVRRSPTPDGNSLLGGVAQLCHAFFHCSPTPELSSHPDELCLRVACDPAGRKCETKGVVVVAALRDRAGDLRFLSRYSNCPLSSHAEEYVVRDEELVRAVMEMAPEDDARSSTKTPGSAGTLTLYQRLQPCHGSSDNRGPLWSCSDALVAGLHRELLGPRGVSLRVAVSYTYRAHWDVRGFESERERRWWGPKVEAAREGIRVFAAAAKDGVTLEALNAEDWAFLVSLCDEDVARDYAAAFGEGGEGFGSKGCGVFTAPAVAHRRAMDEFVAEQIRRHSASGPTNGRATNAAG

SEQ ID NO: 21 - protein, 310 aa, synthetic construct
MADLDDVQDPLLDTALDSTKDEADDSVLSEIAVNDTSVDDGVEDPDHEHKKIAKAGDKVLGNKKEFCGAFYHVPRSKSGCLDKQSCAIAKRGHDATPLTAVALVKYEQQESSEWAIKSVRRYTNCSDKMKHAEEFFLMDIDCQLEARHKGEEGFLDFWNKKKWQITMYLTMQPCHLSTDTGGTKEDQSCCEVMIKAKEKLGDNVEIVIKPTHLCQVGWYKGKPREKPKNAEKGVRKLFKTTGIELECMKEGDWKYLLQYAQPEVENKLPDYDTSRRKTEDEKIGEELHNQQLEQLAPELAQLSVNEKRRK

SEQ ID NO: 22 - protein, 152 aa, synthetic construct
MVYSMDQKNKVTEKLKEGGYSFVLYKDGEWSTSEKRGIAPIMELLKENKELLRGAYVADKVIGKAAALLLIEGGISYLHAEIISEHAIEVLQNSNIEYEYQELVPYIVNRSGDGMCPMEETVLDVTDTKIAFELLQEKIKKMQAAMQAQNMK

SEQ ID NO: 23 - protein, 178 aa, synthetic construct
MISDAAVAGIASKMAEKYYSACKKLSRSIPISTLGVIGKPVPEYSCDGIVPYNSTDLGRMAYKARVEAGFGIFGGRNVAVARVPGWDDPKTGDLVVGFSQGNGFHAEDHVLEQLTKKDISPKKITELYSERQPCAACGPNLENHLSPGTEITWSVQWGSDLEMNSAFTELLGKLIQQQ

SEQ ID NO: 24 - protein, 144 aa, synthetic construct
MAPDSLVWFDPLGLIVLQQVPYNDHPLFGAVSEFIQGKSRSDLRGRNVAAVLLDDGTVIVRASEGGGNHAERVLMGLSEVDPAKVVAVYTERSPCTGRINCHDLLDSSLGADVPVYYTHEMIRGQEGKTAQQIEADRNQFCRGG

SEQ ID NO: 25 - protein, 1368 aa, synthetic construct [sequence omitted]

SEQ ID NO: 26 - protein, 1368 aa, synthetic construct
MDKKYSIGLAIGTNSVGWAVITDEYKVPSKKFKVLGNTDRHSIKKNLIGALLFDSGETAEATRLKRTARRRYTRRKNRICYLQEIFSNEMAKVDDSFFHRLEESFLVEEDKKHERHPIFGNIVDEVAYHEKYPTIYHLRKKLVDSTDKADLRLIYLALAHMIKFRGHFLIEGDLNPDNSDVDKLFIQLVQTYNQLFEENPINASGVDAKAILSARLSKSRRLENLIAQLPGEKKNGLFGNLIALSLGLTPNFKSNFDLAEDAKLQLSKDTYDDDLDNLLAQIGDQYADLFLAAKNLSDAILLSDILRVNTEITKAPLSASMIKRYDEHHQDLTLLKALVRQQLPEKYKEIFFDQSKNGYAGYIDGGASQEEFYKFIKPILEKMDGTEELLVKLNREDLLRKQRTFDNGSIPHQIHLGELHAILRRQEDFYPFLKDNREKIEKILTFRIPYYVGPLARGNSRFAWMTRKSEETITPWNFEEVVDKGASAQSFIERMTNFDKNLPNEKVLPKHSLLYEYFTVYNELTKVKYVTEGMRKPAFLSGEQKKAIVDLLFKTNRKVTVKQLKEDYFKKIECFDSVEISGVEDRFNASLGTYHDLLKIIKDKDFLDNEENEDILEDIVLTLTLFEDREMIEERLKTYAHLFDDKVMKQLKRRRYTGWGRLSRKLINGIRDKQSGKTILDFLKSDGFANRNFMQLIHDDSLTFKEDIQKAQVSGQGDSLHEHIANLAGSPAIKKGILQTVKVVDELVKVMGRHKPENIVIEMARENQTTQKGQKNSRERMKRIEEGIKELGSQILKEHPVENTQLQNEKLYLYYLQNGRDMYVDQELDINRLSDYDVDHIVPQSFLKDDSIDNKVLTRSDKNRGKSDNVPSEEVVKKMKNYWRQLLNAKLITQRKFDNLTKAERGGLSELDKAGFIKRQLVETRQITKHVAQILDSRMNTKYDENDKLIREVKVITLKSKLVSDFRKDFQFYKVREINNYHHAHDAYLNAVVGTALIKKYPKLESEFVYGDYKVYDVRKMIAKSEQEIGKATAKYFFYSNIMNFFKTEITLANGEIRKRPLIETNGETGEIVWDKGRDFATVRKVLSMPQVNIVKKTEVQTGGFSKESILPKRNSDKLIARKKDWDPKKYGGFDSPTVAYSVLVVAKVEKGKSKKLKSVKELLGITIMERSSFEKNPIDFLEAKGYKEVKKDLIIKLPKYSLFELENGRKRMLASAGELQKGNELALPSKYVNFLYLASHYEKLKGSPEDNEQKQLFVEQHKHYLDEIIEQISEFSKRVILADANLDKVLSAYNKHRDKPIREQAENIIHLFTLTNLGAPAAFKYFDTTIDRKRYTSTKEVLDATLIHQSITGLYETRIDLSQLGGD

SEQ ID NO: 27 - protein, 84 aa, synthetic construct
MTNLSDIIEKETGKQLVIQESILMLPEEVEEVIGNKPESDILVHTAYDESTDENVMLLTSDAPEYKPWALVIQDSNGENKIKML

SEQ ID NO: 28 - protein, 125 aa, synthetic construct
MSLPEYDGTTTHGVLVLDDGTQIGFTSGNGDPRYTNYRNNGHVEQKSALYMRENNISNATVYHNNTNGTCGYCNTMTATFLPEGATLTVVPPENAVANNSRAIDYVKTYTGTSNDPKISPRYKGN

SEQ ID NO: 29 - protein, 147 aa, synthetic construct
MEDFHTYHVGKCRLLVHNANCNQEKPVLPKYDGKTTEGVMVTPDGKQISFKSGNSSTPSYPQYKAQSASHVEGKAALYMRENGINEATVFHNNPNGTCGFCDRQVPALLPKGAKLTVVPPSNSVANNVRAIPVPKTYIGNSTVPKIK

SEQ ID NO: 30 - protein, 121 aa, synthetic construct
MLSSSYNAFALTYGVLILDDGKQYSFNSGKPDPIYRNYIPASHVEGKAAIYMRENKIQSGTVYHNNTDGTCPYCDKMLPTLLEKDSTLKVVPPQNATSSKKGWITNEKIYIGNDKIPKTAR

SEQ ID NO: 31 - protein, 144 aa, synthetic construct
MGGDEEEENLTSNNEKKKNANKQKIELPPYDGKTTYGVLILDDGKQYSFNSGKPAPIYRNYIPASHVEGKAAIYMRENKIQSGTVYHNNTDGTCPYCDKMLPTLLEKDSTLKVVPPQNATSSKKGWITNEKIYIGNDKIPKTAR

SEQ ID NO: 32 - protein, 137 aa, synthetic construct
MALLREAYPSMEGATLPPFDGKTTIGLMFYTDASGQYQVKKLFSGEKVLSNYDATGHVEGKAALIMRNEKITEAVVMHNHPSGTCNYCDKQVETLLPKNATLRVIPPENAKAPTSYWNDQPTTYRGDGKDPKAPSKK

SEQ ID NO: 33 - protein, 165 aa, synthetic construct
MIGLMGGLNLYQYAPNSIAWTDWWGLAGSYTLGSYQISAPQLPAYNGQTVGTFYYVNGAGGLESRTFSSGGPTPYPNYANAGHVEGQSALFMRDNGISDGLVFHNNPEGTCGFCVNMTETLLPENSKLTVVPPEGAIPVKRGATGETRTFTGNSKSPKSPVKGEC

SEQ ID NO: 34 - protein, 131 aa, synthetic construct
MQDNTNIIDNRPKLPDYDGKTTHGILVTPNSEHIPFSSGNPNPNYKNYIPASHVEGKSAIYMRENGITSGTIYYNNTDGTCPYCDKMLSTLLEEGSVLEVIPPINAKAPKPSWVDKPKTYIGNNKVPKPNK

SEQ ID NO: 35 - protein, 134 aa, synthetic construct
MGKSLSESQATLSVAQRLLATIGEEGKTAGVLELDGELIPLVSGKSSLPNYAASGHVEGQAALIMRDRGATSGRLLIDNPSGICGYCKSQVATLLPENATLQVGTPLGTVTPSSRWSASRTFTGNDRDPKPWPR

SEQ ID NO: 36 - protein, 148 aa, synthetic construct
MASPAVGTNAAGSSGKNVRMPRDYASELPEYDGKTTHGVLVTNEGKVIQLRSGGKEEPYTGYKAVSASHVEGKAAIWIRENGSSGGTVYHNNTTGTCGYCNSQVKALLPEGVELKIVPPTNAVAKNAQARAVPTINVGNGTQPGRKQK

SEQ ID NO: 37 - protein, 129 aa, synthetic construct
MQGTSSDTIAEMLNSASQPGRTAGVLDIDGELTPLTSGRPSLPNYIASGHVEGQAAMIMRQQQVQSATVYHDNPNGTCGYCYSQLPTLLPEGAALDVVPPAGTVPPSNRWHNGGPSFIGNSSEPKPWPR

SEQ ID NO: 38 - protein, 131 aa, synthetic construct
MGVAGGAATNADAQALLGSIRQAGKTAGVLNIDGDLMPLVSRKSSLPNYAASGHVEGQAALIMRERGVSSAELLIDNPNGICSYCTSQVPTLLPEGAQLMVRPPLGTVPTQWWFNGRTFLGNAANPKPSPW

SEQ ID NO: 39 - protein, 131 aa, synthetic construct
MHNINGCGPSAVQQLLSANGEPGKTAGVLDLNGELTSLVSGKGELPNYAASGHVEGQAAMMMRAEKATSATLYIDNPNGICGYCRSQIATLLPEGATLEVVTPLGTVEPTARWSSSKVFTGNERYPKGWVE

SEQ ID NO: 40 - protein, 153 aa, synthetic construct
MGSAVVGGGIAATGAKALTTGKKLTESPGTLNAAQRLLASIGEEGKTAGVLEVDGALFPLVSGKSVLPNYAASGHVEGQAALLMQGMGATNGRLLIDNPNGICGYCTSQVPTLLPENAVLEVGTPLGTVTPSARWSASKPFIGNDREPKPWPR

SEQ ID NO: 41 - protein, 178 aa, synthetic construct
MDPIRLSGGLNLYQYAPETNNWIDPLGCSGHRRRHEKMPPEGAPLTTGNLFRHAQDEGIPPIFSRKDDEFYHRLIEIYAGTGVLNAYIRGIASHVEPKAGLILNEDGNGWKIGSLYINYPDGPCPGCRRLMPFILNDGSILYVTFPTLGLDGYSYGHFHGGVSGFFREGTPCNLRHPE

SEQ ID NO: 42 - protein, 172 aa, synthetic construct
MPGGGEINRPPTTQADDVPQPVGSEWERTEPDALPGTVRAAVERLQPRPAGSTRPTLGVFNGEEITSGGGDRSLAADLDHDPLRGPPVTFYDHVESKAAARMRRTGSTESDLAIDNTVCGTNDRDQSYPWTCDKILPAILPNGSRLRVWVTRDGGVTWWHRVYIGTGERITK

SEQ ID NO: 43 - protein, 174 aa, synthetic construct
MSPKKPTASSDLKAIGERLGLKPCEGLLGTLPAMKPNSGQRTRGRWHKHPDRELTSGANDRDWEHVKDFWHHNIWSGTAEDTEPRWLAHLELKFAMTMRRTRTKSEPVDQVHEEITINHPDGPCPQCQLLLPYFLEEGSSLTIHWPAGSATYIGRPYFDRPLRDVKPYINEEQQ

SEQ ID NO: 44 - protein, 178 aa, synthetic construct; identical to SEQ ID NO: 41

SEQ ID NO: 45 - protein, 178 aa, synthetic construct
MDPIRLSGGLNLYQYAPETNNWIDPLGCSGYRRRHEKMPPEGARLTTGNLFRHAQDEGIPPIFSSENDEFYYRLIKIYAGTGILNANIRGIASHVEPKAGLILNEDGSGWKIGSLYINYPNGPCLDCRRLMPFILNEGSILYVTFPTLGLDGYSYGHFHGREPGFFREGTPCNLRHPE

SEQ ID NO: 46 - protein, 144 aa, synthetic construct; identical to SEQ ID NO: 24

SEQ ID NO: 47 - protein, 162 aa, synthetic construct; identical to SEQ ID NO: 15

SEQ ID NO: 48 - protein, 206 aa, synthetic construct; identical to SEQ ID NO: 13

SEQ ID NO: 49 - protein, 210 aa, synthetic construct; identical to SEQ ID NO: 16

SEQ ID NO: 50 - protein, 158 aa, synthetic construct
MEGGGPGAVPEGGDGPPAVPAEEVERLRGELPPPVVPGTGQKTHGRWIGPDGRVRAIVSGRDEDAALVHAQLAAKGIPDEPTRNSDVEQKLAAHMVANGIRHVTLVINHRPCRGFDDSCDTLVPIILPEGCTLTVHGQTDKGMRVRVRYTGGARPWWS

SEQ ID NO: 51 - protein, 141 aa, synthetic construct
MDPKKQNPACYQGLAPRQKGKPVRGNLFFPDGRRWNDVALESSRGEPAFDLNIIKPEYRSLSPARGHLEGNVAAWMRSTFHQEMVLYINESPCRKHGKGCLYTLEHFLPRGYVLHVWSRNDRGEWRGNTFRGSGEAFTEGA

SEQ ID NO: 52 - protein, 143 aa, synthetic construct
MCPIWVKNALQELVGRKETSGKVFDVDGKPIGPDIQSGYKDRELRRGVYETLRKSPFFQKHFPSTATWYVSLHVEAQYAVWMLRNRIKHATVVINNTYVCSDMNRLHDNCMTAVPHILPEGYTMTVWKADRTEVTLRGKAPKE

SEQ ID NO: 53 - protein, 143 aa, synthetic construct
MPASKPSRFKPMRTDPAKADEIRPHVGKDRAVATLWDADGNRVLGLHSADDDGPAATAAWKPPWRDYVRLRRHVEAHAAARMHQDGHKTMVMYINLPPCKYFDGCKLNLEDILPKGSTLWMHRVFQNGGTKIYQFNGTGRAYV

SEQ ID NO: 54 - protein, 142 aa, synthetic construct
MPGANGSERVDELAERLPPTVVPNTSAKTHGWWFTGQGAAQELISGEGPDARAAYEALREEGYPRPGMPFVAMHVEIKLAAHMRRNDIEHATVVINNIPCPLVWGCENLIGVVLPEGSSLTVHGSNGYERTFTGGRKPPWPR

SEQ ID NO: 55 - protein, 138 aa, synthetic construct
MPRRFNPACWQGLKPYDQAGTAEGNLFIAPGKRWNTRPMQASKLEVGPQSDLHPQWRSRKAPWHIEGKIAAYMRQKGFTDGCVYLNARPCSGPDGCARNLPDLLPVGSTLHVHARYIDRTGETRFYYREYRGTGKALT

SEQ ID NO: 56 - protein, 138 aa, synthetic construct
MGLEGTPCDGFGALAARRKSLGLPAAGSEGDTSTLSLLRINGQSFEGINSSDQNPKTPITLDRVNAQTKTHAEAEAVQKAVNAGMAGKASHAEMWVDRDPCRACGIPGAGGLRSLARNLGCPITVHSPSGTQVYTPTK

SEQ ID NO: 57 - protein, 182 aa, synthetic construct
MLGPPLDLNPANRAPEFGRCDGTSWIDSYRTINNATDLFGRPVWPNHRGTVAVARIDGDIYFGVNSKAPGYSDADWNLAAGLRDQMALEHPELIRGESRGSRPLDAVFHAEANLLIRASRYVGSLVKRSIEVQVDRPVCWSCEQALPKVGLELGDPYVTIREVRSGRASVMWQGEWLVWRKK

SEQ ID NO: 58 - protein, 152 aa, synthetic construct
MGWVDPLGLVSGGAWDAISFFRDQNSLLSVVDEDLLAASGAKNAQNTVALLRVGDREFIGVNSRIQNPKNPFTAGPINNITKFHAEGNAAQQAIDAGMVGKHRIAEMWVDRDLCHACGPSNGVGSLTRALGLDAIIVHTPAGTRKFNAPCAG

SEQ ID NO: 59 - protein, 181 aa, synthetic construct
MVKGLDGFVKTCTRTRGKLTARASTAVGGCPVGLVAYNSEEMSHWAYRYRTESEYFEGDHNVAVAKVPGWNDPRTGDFIIANSKFSGHSETEILGKLEAKGFTPGQITALYTERQPCPACASVLTGSLKEGTPVTWSVPYHPDYAKESRSLLDSYVRQANGQQRARPTTTQRLTEGNEAHD

SEQ ID NO: 60 - protein, 129 aa, synthetic construct
MRLGQSVDPRLLEMAKEARVTQAGISREAFASYNVATARVRVGTEIRYLDAGNSPGRLMHSEDWLITQVEELRRVHGRESVALEQLFSERIPCGECLPKLERLFNAEVFYAVAKRGTRATDLMKAYGLR

SEQ ID NO: 61 - protein, 167 aa, synthetic construct
MPDPLGLAPAANDRAYVPNPLTWADPYGLACTGTTEPGSTDLSQAVIQERLRLGKKGNNFAAARYIDDNGVEQIAVAASSKGQFMHAERKLVRQYGDKITEVYSEFEPCIGTNQCRKTLGDMGIKYTYSWAWTLSKDGVAANAARKAYVDQIFDDAEAGNWAAPWAD

SEQ ID NO: 62 - protein, 150 aa, synthetic construct
MNIDGDSYLVPGALAAMFLHKPGRGGKGKVGYGTTDLGQSVRLQRLIDKNRGMTNYAAARLDDGDVIVGKSKKHVHAEEHLFQQAGKRKIVELYSEREPCSNKCEDLVKDIPFVSWSFKWNHPDRIKQDAIRDKANADLKDAVRSLFNSP

SEQ ID NO: 63 - protein, 162 aa, synthetic construct
MQGYIVDESGRVLDANGLPIASLPPADDLSKWANYTVESGLHDDLAALENRLDLLYRQQFGLPMAPPAWHLETQLAYRVATREVALRDSTLRLVMNNPGGVCDAVPLTGTGPDRQRQAVAGCIQAVKMLLPAGTTMIIYYPDPDDPAELLEITVRGVGRWLD

SEQ ID NO: 64 - protein, 229 aa, synthetic construct [sequence omitted]

SEQ ID NO: 65 - protein, 138 aa, synthetic construct
GSYALGPYQISAPQLPAYNGQTVGTFYYVNDAGGLESKVFSSGGPTPYPNYANAGHVEGQSALFMRDNGISEGLVFHNNPEGTCGFCVNMTETLLPENAKMTVVPPEGAIPVKRGATGETKVFTGNSNSPKSPTKGGC

SEQ ID NO: 66 - protein, 140 aa, synthetic construct
MDGPHGTPVLDRIAKLREELPPPAVPGKGQKTDGRWFDGNGAVRDSVSGKDVDSEEAWRLLRESGIPLPRPPVVAHAEMKVAAAMRRLNVRHAVLVITNVPCDERWSCENLLPAVLPVGCSLSVHGPGYQRTFHGRTPKW

SEQ ID NO: 67 - protein, 164 aa, synthetic construct
MRPTTPPGPHARWRPDPPSAPHVAAIRRVGWPKKPQSDDDVRARGQLYHRDGTPWNASMLIASRRGPASQRTDLKEPWASDPGYTTGWHIEGNTAALMVKHQQRDAVLYINQAVCGAEEPQDPKRCHSNIVAMLSVGYALYVHSVQESGWLRRRVYKGTGEAIR

SEQ ID NO: 68 - protein, 120 aa, synthetic construct
MQRHGGRVRLLSGENDDPHSWQQQAARFLRETFPDKGPGLAVLSRHVEIQLAVRLRHRPTNEVVHEVLVIDRVVCGRDPRTQGREYTCDTVLPFVLDEGATLTVVEHDGARVTYRGRGRR

SEQ ID NO: 69 - protein, 95 aa, synthetic construct
MKILYIKSAEGYPSLMLKNNPRIPTNARSYTHVEGRAASIMRQSGIKSAKLTINNTNGVCDPCRGNMEKSLLPDGGKLNVRYPDGQGGYTQRILI

SEQ ID NO: 70 - protein, 106 aa, synthetic construct
MREFGLPIEPPAWHLETQLAYRVSKREVALRENTLRLVMNNPGGVCDAVPAKDRGPDGQRQVVAGCVQAIQMLLPAGTTMIIYYPDPANPAKLLQVTVRGVGRWLD

SEQ ID NO: 71 - protein, 123 aa, synthetic construct
MLQGWRLAVGDGSSDRELASGTKLASGQTDPSYTAAVQRARELGLARGGFVPDIARHIEIKEASTMTAGETRTIVIGKDPCGIDPVTNVSCHPFLRYFLPPGATLIVYGPRGEPYRYEGKRTS

SEQ ID NO: 72 - protein, 113 aa, synthetic construct
MVGATTDSVPTQPGGRARSAPPRPPRPGKTHGRWCDSDGNAVVLESGKGGEYYEATRARGVALGLAKGIPNAEPSIARHVETQFVSRMIDQGIEYAEIEINRPVCGTTPKDQQ

SEQ ID NO: 73 - protein, 162 aa, synthetic construct; identical to SEQ ID NO: 63

SEQ ID NO: 74 - protein, 162 aa, synthetic construct; identical to SEQ ID NO: 63

SEQ ID NO: 75 - protein, 135 aa, synthetic construct
MGAPRTMGNMGVAQISIPGVQSKMAASSQIPDPTAAQRALGFVGEVNETFPSASVWTGGDTPYLLNRKVDSEAKILNNIAAQLGDNTSASGTINLFTERPPCESCSNTIIKFQEKYPNIKINVMDSNGVIRPSKR

SEQ ID NO: 76 - protein, 184 aa, synthetic construct
MGQGFDGVQPANEFIKAWGEAMVAEAAGLGIVAGLGRFGLWGAKGATPVVTAEGRIGNSVFTDVNQTARPAAQANPNQPTLIADRVDAKIAAKGTPHPNGNMADAHAEIGVIQKAFNEGKTVGSDMTMNVVGKDVCGYCRGDIAAAASKSGLKSLTIQAKDDITGLPKTYYWEVGMKSIREKKI

SEQ ID NO: 77 - protein, 179 aa, synthetic construct
MYLPRGTSVTSKETVAKDPVSLAGQADNEAGILVDRNVIVGGTKGVSPVVTAEGKIGGKTFTDFNQTARPASEANASQPTLISDRVTAKADASGKVLPNGNMADAHAEIGVIQQAYTAGKTMGASMELTVSGKAVCGYCRGDIAAMAEKSGLTSLEVKEVATGKTLYWQPGMRALRERN

SEQ ID NO: 78 - protein, 167 aa, synthetic construct
MKKPTGSIVSPETTIVQESSKILDKKTHTSIPKVEAELIDKETGKIFKDTNQGNRPDYFLGDKSRPTLINDRIEAKVEKNPSKYLPNGNMASAHAEVGTIQQAFEDGITVGRDMNMKVTKEAVCGYCRGDIAAMADKAGLKSLTVYEESTGKTLYWNPGMKSLKEKK

SEQ ID NO: 79 - protein, 172 aa, synthetic construct
MAGVLAPEVYLAKTPRVGDNSARGVGDGRSTTPKVTAEAEVDGVKFNDTNQNARPSEAANPNIPTLISDDIQVKIDKNPDKPFPNGNMATAHAEVGAIQQAYDAGKTQGKNMTMRVTGEDVCDYCRSDLRKAADKSGLNSLSVYEETTGRTLTWTRREDGTIGKVKIIEPEG

SEQ ID NO: 80 - protein, 176 aa, synthetic construct
MGVDRKTAQGYAETKQGMDTIVASVTPILGAAAAKQLSKVVDANIKVVAEGNVNGAKFSDTNQGARPSNLADVNKPTLIDGRIQAKIDKQNKPLPNGNMATAHAEVGVIQQAFEKGMSQGREMTMSVSKEPVCGYCRSDIAAMADKAGLKSLTIYEETTGSVLYWQPGMKSLKIRD

SEQ ID NO: 81 - protein, 178 aa, synthetic construct
MDRQTAESYTETKQGLEIIAASVTPILGSVAAKQLSKIVDANLKVVARGNVDGARFSDTNQGVRPSQLADFNKPTLINDVVQAKIDKRPDKNYPNGNMGTAHAEVGVIQQAFDKGMTQGREMAMSVGGKEVCNYCLSDVRIMAEKAGLKSLTIYEEATGNVLFWQQGMKKIENRGPAK

SEQ ID NO: 82 - protein, 207 aa, synthetic construct
MTKSALGEIVIVVSDLVIPTNYVEILPVGKLSKVAKILKIGEDGTKSAGRLAEELAELQKVDIKFGKTLPGAKAPITVTAESNIGGKHMFDTNQTARPEVNRTNTPTLAAGNAKIDPSNPNLTMKNAHAEIALIQRAYDAGLTKGETMQVLVRGKEVCDHCGQVMKTMYERSGLSKLIIHDTTSGTTTTYYKVIDAKTKIATTKIEV

SEQ ID NO: 83 - protein, 144 aa, synthetic construct
MDDSYYMKQALLEAQKAGERGEVPVGAVVVCKDRIIARAHNLTETLTDVTAHAEMQAITAAASTLGGKYLNECALYVTVEPCVMCAGAIAWAQTGKLVFGAEDEKRGYQRYAPQALHPKTMVVKGVLADECAALMKNFFAAKRK

SEQ ID NO: 84 - protein, 207 aa, synthetic construct; identical to SEQ ID NO: 82

SEQ ID NO: 85 - DNA, 16 bp, synthetic construct
  source 1..16: mol_type = other DNA
aggcaggccattccca

SEQ ID NO: 86 - DNA, 16 bp, synthetic construct
  source 1..16: mol_type = other DNA
tccgtccggtaagggt

SEQ ID NO: 87 - DNA, 20 bp, synthetic construct
  source 1..20: mol_type = other DNA
tcgccgtacgcggacaaggg

SEQ ID NO: 88 - DNA, 20 bp, synthetic construct
  source 1..20: mol_type = other DNA
agcggcatgcgcctgttccc

SEQ ID NO: 89 - DNA, 23 bp, synthetic construct
  source 1..23: mol_type = other DNA
gaacacaaagcatagactgcggg

SEQ ID NO: 90 - DNA, 23 bp, synthetic construct
  source 1..23: mol_type = other DNA
cttgtgtttcgtatctgacgccc

SEQ ID NO: 91 - DNA, 23 bp, synthetic construct
  source 1..23: mol_type = other DNA
cagcagtatggtgcgctgtgcgg

SEQ ID NO: 92 - DNA, 23 bp, synthetic construct
  source 1..23: mol_type = other DNA
gtcgtcataccacgcgacacgcc

SEQ ID NO: 93 - DNA, 24 bp, synthetic construct
  source 1..24: mol_type = other DNA
acaaggatcccagccccgtgaagg

SEQ ID NO: 94 - DNA, 29 bp, synthetic construct
  source 1..29: mol_type = other DNA
tctcagcatagcactcaatgcggtctggg

SEQ ID NO: 95 - DNA, 23 bp, synthetic construct
  source 1..23: mol_type = other DNA
tagcacccatgacaatgacatgg

SEQ ID NO: 96 - DNA, 23 bp, synthetic construct
  source 1..23: mol_type = other DNA
gaccagccagcgtctggcgccgg

SEQ ID NO: 97 - DNA, 26 bp, synthetic construct
  source 1..26: mol_type = other DNA
ctagcacatgagagaacaatattggg

SEQ ID NO: 98 - DNA, 24 bp, synthetic construct
  source 1..24: mol_type = other DNA
gcacacacacactagtacctctgg

SEQ ID NO: 99 - DNA, 28 bp, synthetic construct
  source 1..28: mol_type = other DNA
acaaagtacaaacggcagaagctggagg

SEQ ID NO: 100 - DNA, 27 bp, synthetic construct
  source 1..27: mol_type = other DNA
actggaacacaaagcatagactgcggg

SEQ ID NO: 101 - DNA, 28 bp, synthetic construct
  source 1..28: mol_type = other DNA
cctggcagcagtatggtgcgctgtgcgg

SEQ ID NO: 102 - DNA, 27 bp, synthetic construct
  source 1..27: mol_type = other DNA
gcaaccaacccgaccaagaaatgcagt

SEQ ID NO: 103 - DNA, 27 bp, synthetic construct
  source 1..27: mol_type = other DNA
agtcattcaacgtcacaaccaccaggt

SEQ ID NO: 104 - DNA, 23 bp, synthetic construct
  source 1..23: mol_type = other DNA
tctccatcgacgcaccgccgggg

SEQ ID NO: 105 - DNA, 23 bp, synthetic construct
  source 1..23: mol_type = other DNA
caggtcccccgccggatgatcgg

SEQ ID NO: 106 - DNA, 23 bp, synthetic construct
  source 1..23: mol_type = other DNA
gatccattactgggaatcatcgg

SEQ ID NO: 107 - DNA, 23 bp, synthetic construct
  source 1..23: mol_type = other DNA
aagcgctatattgtgaaaaatgg

SEQ ID NO: 108 - DNA, 27 bp, synthetic construct
  source 1..27: mol_type = other DNA
caatgcgtcctttgacagcagctgtgg

SEQ ID NO: 109 - DNA, 30 bp, synthetic construct
  source 1..30: mol_type = other DNA
cataagcgctatattgtgaaaaatggggca

SEQ ID NO: 110 - DNA, 30 bp, synthetic construct
  source 1..30: mol_type = other DNA
cataagtgctatattgtgaaaaatggggca